European Patent Application EP 4 644 563 A1, published November 5, 2025. Title: 原位测序文库的构建方法、原位测序方法及应用. Applicant: 深圳华大生命科学研究院. Application CN. The sequence listing filed with the application follows.

SEQUENCE LISTING (6 sequences)

SEQ ID NO: 1 - DNA, 95 bp, synthetic construct
  source 1..95: mol_type = other DNA
cctgcttggaggaggtggaactgattcctttgactcacattgcgtcctatcttctttggagcctgtctatttagttagtgggccagcgtcttggc

SEQ ID NO: 2 - DNA, 95 bp, synthetic construct
  source 1..95: mol_type = other DNA
ggattttggccggcgcagtgctgattcctttgactcacattgcgtcctatcttctttggagcctgtctatttagtcgggactacatgggctggat

SEQ ID NO: 3 - DNA, 95 bp, synthetic construct
  source 1..95: mol_type = other DNA
agccttctccgctggaactcctgattcctttgactcacattgcgtcctatcttctttggagcctgtctatttagtcctcaacttagctggactgc

SEQ ID NO: 4 - DNA, 95 bp, synthetic construct
  source 1..95: mol_type = other DNA
ggcagtcctagctgctggcgctgattcctttgactcacattgcgtcctatcttctttggagcctgtctatttagtgtatgtctgtgcgtggtgat

SEQ ID NO: 5 - DNA, 95 bp, synthetic construct
  source 1..95: mol_type = other DNA
ttgagtatctatttattaagctgattcctttgactcacattgcgtcctatcttctttggagcctgtctatttagtcgcctctaatgtctgacgtt

SEQ ID NO: 6 - DNA, 20 bp, synthetic construct
  source 1..20: mol_type = other DNA
gtcctatcttctttggagcc